European Patent Specification EP 3 298 030 B1, published January 18, 2023. Title: Anti-Cancer fusion polypeptide. Applicant: Pieris AG. The sequence listing filed with the application follows.

SEQUENCE LISTING (75 sequences)

SEQ ID NO: 1 - protein, 156 aa, artificial
  wildtype Tlc
HHLLASDEEIQDVSGTWYLKAMTVDREFPEMNLESVTPMTLTTLEGGNLEAKVTMLISGRCQEVKAVLEKTDEPGKYTADGGKHVAYIIRSHVKDHYIFYCEGELHGKPVRGVKLVGRDPKNNLEALEDFEKAAGARGLSTESILIPRQSETCSPG

SEQ ID NO: 2 - protein, 178 aa, artificial
  Wildtype NGAL
QDSTSDLIPAPPLSKVPLQQNFQDNQFQGKWYVVGLAGNAILREDKDPQKMYATIYELKEDKSYNVTSVLFRKKKCDYWIRTFVPGCQPGEFTLGNIKSYPGLTSYLVRVVSTNYNQHAMVFFKKVSQNREYFKITLYGRTKELTSELKENFIRFSKSLGLPENHIVFPVPIDQCIDG

SEQ ID NO: 3 - protein, 178 aa, artificial
  NGAL98 control
QDSTSDLIPAPPLSKVPLQQNFQDNQFHGKWYVVGLAGNAILREDKDPQKMYATIYELKEDKSYNVTSVLFRKKKCDYWIRTFVPGSQPGEFTLGNIKSYPGLTSYLVRVVSTNYNQHAMVFFKKVSQNREYFKITLYGRTKELTSELKENFIRFSKSLGLPENHIVFPVPIDQCIDG

SEQ ID NO: 4 - protein, 178 aa, artificial
  Lipocalin mutein
QDSTSDLIPAPPLSKVPLQQNFQDNQFHGKWYVVGVAGNAMLREDKDPLKMRATIYELKEDKSYNVTGVSFWRKKCHYKIGTFVPGSQPGEFTLGDIKSGPGQTSNLVRVVSTNYNQHAMVFFKEVRQNREWFAITLYGRTKELTSELKENFIRFSKSLGLPENHIVFPVPIDQCIDG

SEQ ID NO: 5 - protein, 178 aa, artificial
  Lipocalin mutein
QDSTSDLIPAPPLSKVPLQQNFQDNQFHGKWYVVGRAGNVALREDKDPPKMRATIYELKEDKSYNVTNVRFAMKKCMYSIGTFVPGSQPGEFTLGQIKSEPGNTSNLVRVVSTNYNQHAMVFFKEVYQNREIFFITLYGRTKELTSELKENFIRFSKSLGLPENHIVFPVPIDQCIDG

SEQ ID NO: 6 - protein, 178 aa, artificial
  Lipocalin mutein
QDSTSDLIPAPPLSKVPLQQNFQDNQFQGKWYVVGVAGNALLREDKDPLKMRATIYELKEDKSYDVTVVSFWRKKCHYKIGTFVPGSQPGEFTLGDIKSGPGQTSNLVRVVSTNYNQHAMVFFKEVRQNREWFAITLYGRTKELTSELKENFIRFSKSLGLPENHIVFPVPIDQCIDG

SEQ ID NO: 7 - protein, 178 aa, artificial
  Lipocalin mutein
QDSTSDLIPAPPLSKVPLQQNFQDNQFQGKWYVVGVAGNVRLREDKDPPKMRATIYELKEDKSYDVTGVSFRGKKCHYKIGTFVPGSQPGEFTLGDIKSGPGETSNLVRVVSTNYNQHAMVFFKEVRQNREWFFITLYGRTKELTSELKENFIRFSKSLGLPENHIVFPVPIDQCIDG

SEQ ID NO: 8 - protein, 178 aa, artificial
  Lipocalin mutein
QDSTSDLIPAPPLSKVPLQQNFQDNQFQGKWYVVGVAGNGMLREDKDPLKMRATIYELKEDKSYDVTSVAFRNKKCHYKIGTFVPGSQPGEFTLGQIKSGPGETSNLVRVVSTNYNQHAMVFFKEVRQNREWFFITLYGRTKELTSELKENFIRFSKSLGLPENHIVFPVPIDQCIDG

SEQ ID NO: 9 - protein, 178 aa, artificial
  Lipocalin mutein
QDSTSDLIPAPPLSKVPLQQNFQDNQFQGKWYVVGRAGNVGLREDKDPPKMWATIYELKEDKSYDVTNVRFARKKCLYSIGTFVPGSQPGEFTLGQIKSEPGNTANLVRVVSTNYNQHAMVFFKEVYQNREIFFIILYGRTKELTSELKENFIRFSKSLGLPENHIVFPVPIDQCIDG

SEQ ID NO: 10 - protein, 178 aa, artificial
  Lipocalin mutein
QDSTSDLIPAPPLSKVPLQQNFQDNQFQGKWYVVGRAGNVGLREDKDPPKMWATIYELKEDKSYDVTNVRFARKKCTYSIGTFVPGSQPGEFTLGQIKSEPGGTANLVRVVSTNYNQHAMVFFKEVYQNREIFFIILYGRTKELTSELKENFIRFSKSLGLPENHIVFPVPIDQCIDG

SEQ ID NO: 11 - protein, 178 aa, artificial
  Lipocalin mutein
QDSTSDLIPAPPLSKVPLQQNFQDNQFQGKWYVVGRAGNGALREDKDPPKMWATIYELKEDKSYDVTNVRFARKKCVYSIGTFVPGSQPGEFTLGPIKSEPGNTASLVRVVSTNYNQHAMVFFKEVYQNREIFFIILYGRTKELTSELKENFIRFSKSLGLPENHIVFPVPIDQCIDG

SEQ ID NO: 12 - protein, 178 aa, artificial
  Lipocalin mutein
QDSTSDLIPAPPLSKVPLQQNFQDNQFQGKWYVVGRAGNVALREDKDPPKMRATIYELKEDKSYDVTAVRFARKKCLYSIGTFVPGSQPGEFTLGRIKSEPGYTANLVRVVSTNYNQHAMVFFKEVYQNREIFFIILYGRTKELTSELKENFIRFSKSLGLPENHIVFPVPIDQCIDG

SEQ ID NO: 13 - protein, 178 aa, artificial
  Lipocalin mutein
QDSTSDLIPAPPLSKVPLQQNFQDNQFQGKWYVVGRAGNVALREDKDPPKMRATIYELKEDKSYDVTNVVFAGKKCKYSIGTFVPGSQPGEFTLGRIKSPPGNTANLVRVVSTNYNQHAMVFFKEVYQNREIFFIILYGRTKELTSELKENFIRFSKSLGLPENHIVFPVPIDQCIDG

SEQ ID NO: 14 - protein, 178 aa, artificial
  Lipocalin mutein
QDSTSDLIPAPPLSKVPLQQNFQDNQFQGKWYVVGRAGNLGLREDKDPPKMWATIYELKEDKSYDVTNVRFARKKCMYSIGTFVPGSQPGEFTLGQIKSEPGSTANLVRVVSTNYNQHAMVFFKEVYQNREIFFITLYGRTKELTSELKENFIRFSKSLGLPENHIVFPVPIDQCIDG

SEQ ID NO: 15 - protein, 178 aa, artificial
  Lipocalin mutein
QDSTSDLIPAPPLSKVPLQQNFQDNQFQGKWYVVGRAGNVGLREDKDPPKMWATIYELKEDKSYDVTNVRFAGKKVKYTIGTFVPGSQPGEFTLGQIKSEPGNTATLVRVVSTNYNQHAMVFFKEVYQNREIFFITLYGRTKELTSELKENFIRFSKSLGLPENHIVFPVPIDQAIDG

SEQ ID NO: 16 - protein, 178 aa, artificial
  Lipocalin mutein
QDSTSDLIPAPPLSKVPLQQNFQDNQFQGKWYVVGRAGNVGLREDKDPPKMRATIYELKEDKSYDVTGVRFGEKKIKYSIGTFVPGSQPGEFTLGQIKSQPGDTANLVRVVSTNYNQHAMVFFKEVYQNREIFFIILYGRTKELTSELKENFIRFSKSLGLPENHIVFPVPIDQAIDG

SEQ ID NO: 17 - protein, 178 aa, artificial
  Lipocalin mutein
QDSTSDLIPAPPLSKVPLQQNFQDNQFQGKWYVVGRAGNVGLREDKDPPKMRATIYELKEDKSYDVTGVRFDSKKVTYSIGTFVPGSQPGEFTLGQIKSEPGNTANLVRVVSTNYNQHAMVFFKEVYQNREIFFIILYGRTKELTSELKENFIRFSKSLGLPENHIVFPVPIDQAIDG

SEQ ID NO: 18 - protein, 152 aa, artificial
  lipocalin mutein
ASDEEIQDVSGTWYLKAMTVDEGCRPWNIFSVTPMTLTTLEGGNLEAKVTMAIDGPAQEVKAVLEKTDEPGKYTADGGKHVAYIIRSHVKDHYIFYSEGVCDGSPVPGVWLVGRDPKNNLEALEDFEKAAGARGLSTESILIPRQSETSSPG

SEQ ID NO: 19 - protein, 152 aa, artificial
  lipocalin mutein
TSDEEIQDVSGTWYLKAMTVDEGCRPWNIFSVTPMTLTTLEGGNLEAKVTMAIDGPAQEVRAVLEKTDEPGKYTADGGKHDAYIIRSHVKDHYIFYSEGVCDGSPVPGVWLVGRDPENNLEALEDFEKTAGARGLSTESILIPRQSETSSPG

SEQ ID NO: 20 - protein, 152 aa, artificial
  lipocalin mutein
ASDEEIQDVSGTWYLKAMTVDEGCRPWNIFSVTPMTLTTLEGGNLEAKVTMAIDGPAQEVNAVLEKTDEPGKYTADGGKHVAYIIRSHVRDHYIFYSEGVCDGSPVPGVWLVGRDPENNLEALEDFEKTAGARGLSTESILIPRQSETSSPG

SEQ ID NO: 21 - protein, 152 aa, artificial
  lipocalin mutein
VSDEEIQDVSGTWYLKAMTVDEGCRPWNIFSVTPMTLTTLEGGNLEAKVTMAIDGPAQEVRAVLEKTDEPGKYTADGGKHVAYIIRSHVEDHYIFYSEGVCDGSPVPGVWLVGRDPENNLEALEDFEKTAGARGLSTESILIPRQSETSSPG

SEQ ID NO: 22 - protein, 152 aa, artificial
  lipocalin mutein
ASDEEIQDVSGTWYLKAMTVDEGCRPWNIFSVTPMTLSTLEGGNLEAKVTMAIDGPAQEVKAVLEKTDEPGKYTADGGKHVAYIIRSHVKDHYIFYSEGVCDGSPVPGVWLVGRDPKNNLEALEDFEKAAGARGLSTESILIPRQIETSSPG

SEQ ID NO: 23 - protein, 152 aa, artificial
  lipocalin mutein
ASDEEIQDVSGTWYLKAMTVDEGCRPWNIFSVTPMTLTTLEGGNLEAEVTMAIDGPAQEVKAVLEKADEPGKYTADGGKHVAYIIRSHVKDHYIFYSEGVCDGSPVPGVWLVGRDPKNNLEALEDFEKTAGARGLSTESILIPSQIETSSPG

SEQ ID NO: 24 - protein, 152 aa, artificial
  lipocalin mutein
TSDEEIQDVSGTWYLKAMTVDEGCRPWNIFSVTPMTLTTLEDGNLEAKVTMAIDGPAQEVKAVLEKADEPGKYTADGGKHVAYIIRSHVKDHYIFYSEGVCDGSPVPGVWLVGRDPKNNLEALEDFEKAAGARGLSTESILIPRQIETSSPG

SEQ ID NO: 25 - protein, 178 aa, artificial
  lipocalin mutein
QDSTSDLIPAPPLSKVPLQQNFQDNQFHGKWYVVGQAGNIKLREDKDPNKMMATIYELKEDKSYNVTGVTFDDKKCTYAISTFVPGSQPGEFTLGKIKSFPGHTSSLVRVVSTNYNQHAMVFFKFVFQNREEFYITLYGRTKELTSELKENFIRFSKSLGLPENHIVFPVPIDQCIDG

SEQ ID NO: 26 - protein, 178 aa, artificial
  lipocalin mutein
QDSTSDLIPAPPLSKVPLQQNFQDNQFHGKWYVVGQAGNIRLREDKDPIKMMATIYELKEDKSYDVTMVKFDDKKCMYDIWTFVPGSQPGEFTLGKIKSFPGHTSSLVRVVSTNYNQHAMVFFKFVFQNREEFYITLYGRTKELTSELKENFIRFSKSLGLPENHIVFPVPIDQCIDG

SEQ ID NO: 27 - protein, 178 aa, artificial
  lipocalin mutein
QDSTSDLIPAPPLSKVPLQQNFQDNQFHGKWYVVGQAGNIRLREDKDPNKMMATIYELKEDKSYDVTAVAFDDKKCTYDIWTFVPGSQPGEFTLGKIKSFPGHTSSLVRVVSTNYNQHAMVFFKFVFQNREEFYITLYGRTKELTSELKENFIRFSKSLGLPENHIVFPVPIDQCIDG

SEQ ID NO: 28 - protein, 178 aa, artificial
  lipocalin muein
QDSTSDLIPAPPLSKVPLQQNFQDNQFHGKWYVVGQAGNIKLREDKDPNKMMATIYELKEDKSYDVTAVAFDDKKCTYDIWTFVPGSQPGEFTLGKIKSFPGHTSSLVRVVSTNYNQHAMVFFKFVFQNREEFYITLYGRTKELTSELKENFIRFSKSLGLPENHIVFPVPIDQCIDG

SEQ ID NO: 29 - protein, 175 aa, artificial
  lipocalin mutein
QDSTSDLIPAPPLSKVPLQQNFQDNQFHGKWYVVGQAGNIKLREDSKMMATIYELKEDKSYDVTGVSFDDKKCTYAIMTFVPGSQPGEFTLGKIKSFPGHTSSLVRVVSTNYNQHAMVFFKFVFQNREEFYITLYGRTKELTSELKENFIRFSKSLGLPENHIVFPVPIDQCIDG

SEQ ID NO: 30 - protein, 178 aa, artificial
  lipocalin mutein
QDSTSDLIPAPPLSKVPLQQNFQDNQFHGKWYVVGQAGNIKLREDKDPVKMMATIYELKEDKSYDVTGVTFDDKKCRYDISTFVPGSQPGEFTFGKIKSFPGHTSSLVRVVSTNYNQHAMVFFKFVFQNREEFYITLYGRTKELTSELKENFIRFSKSLGLPENHIVFPVPIDQCIDG

SEQ ID NO: 31 - protein, 178 aa, artificial
  lipocalin mutein
QDSTSDLIPAPPLSKVPLQQNFQDNQFHGKWYVVGQAGNIRLREDKDPHKMMATIYELKEDKSYDVTGVTFDDKKCTYAISTFVPGSQPGEFTLGKIKSFPGHTSSLVRVVSTNYNQHAMVFFKFVFQNREEFYITLYGRTKELTSELKENFIRFSKSLGLPENHIVFPVPIDQCIDG

SEQ ID NO: 32 - protein, 178 aa, artificial
  lipocalin mutein
QDSTSDLIPAPPLSKVPLQQNFQDNQFHGKWYVVGQAGNIKLREDKDPNKMMATIYELKEDKSYDVTGVTFDDKKCTYAISTLVPGSQPGEFTFGKIKSFPGHTSSLVRVVSTNYNQHAMVFFKFVFQNREEFYITLYGRTKELTSELKENFIRFSKSLGLPENHIVFPVPIDQCIDG

SEQ ID NO: 33 - protein, 178 aa, artificial
  lipocalin mutein
QDSTSDLIPAPPLSKVPLQQNFQDNQFHGKWYVVGQAGNIRLREDKDPSKMMATIYELKEDKSYDVTAVTFDDKKCNYAISTFVPGSQPGEFTLGKIKSFPGHTSSLVRVVSTNYNQHAMVFFKFVFQNREEFYITLYGRTKELTSELKENFIRFSKSLGLPENHIVFPVPIDQCIDG

SEQ ID NO: 34 - protein, 448 aa, artificial
  antibody heavy chain
QVQLQQWGAGLLKPSETLSLTCAVYGGSFSGYYWSWIRQSPEKGLEWIGEINHGGYVTYNPSLESRVTISVDTSKNQFSLKLSSVTAADTAVYYCARDYGPGNYDWYFDLWGRGTLVTVSSASTKGPSVFPLAPCSRSTSESTAALGCLVKDYFPEPVTVSWNSGALTSGVHTFPAVLQSSGLYSLSSVVTVPSSSLGTKTYTCNVDHKPSNTKVDKRVESKYGPPCPPCPAPEFLGGPSVFLFPPKPKDTLMISRTPEVTCVVVDVSQEDPEVQFNWYVDGVEVHNAKTKPREEQFNSTYRVVSVLTVLHQDWLNGKEYKCKVSNKGLPSSIEKTISKAKGQPREPQVYTLPPSQEEMTKNQVSLTCLVKGFYPSDIAVEWESNGQPENNYKTTPPVLDSDGSFFLYSRLTVDKSRWQEGNVFSCSVMHEALHNHYTQKSLSLSLGK

SEQ ID NO: 35 - protein, 216 aa, artificial
  antibody polypeptide chain
EIVLTQSPATLSLSPGERATLSCRASQSVSSYLAWYQQKPGQAPRLLIYDASNRATGIPARFSGSGSGTDFTLTISSLEPEDFAVYYCQQRSNWPPALTFGGGTKVEIKRTVAAPSVFIFPPSDEQLKSGTASVVCLLNNFYPREAKVQWKVDNALQSGNSQESVTEQDSKDSTYSLSSTLTLSKADYEKHKVYACEVTHQGLSSPVTKSFNRGEC

SEQ ID NO: 36 - protein, 641 aa, artificial
  fusion polypeptide heavy chain
QVQLQQWGAGLLKPSETLSLTCAVYGGSFSGYYWSWIRQSPEKGLEWIGEINHGGYVTYNPSLESRVTISVDTSKNQFSLKLSSVTAADTAVYYCARDYGPGNYDWYFDLWGRGTLVTVSSASTKGPSVFPLAPCSRSTSESTAALGCLVKDYFPEPVTVSWNSGALTSGVHTFPAVLQSSGLYSLSSVVTVPSSSLGTKTYTCNVDHKPSNTKVDKRVESKYGPPCPPCPAPEFLGGPSVFLFPPKPKDTLMISRTPEVTCVVVDVSQEDPEVQFNWYVDGVEVHNAKTKPREEQFNSTYRVVSVLTVLHQDWLNGKEYKCKVSNKGLPSSIEKTISKAKGQPREPQVYTLPPSQEEMTKNQVSLTCLVKGFYPSDIAVEWESNGQPENNYKTTPPVLDSDGSFFLYSRLTVDKSRWQEGNVFSCSVMHEALHNHYTQKSLSLSLGKGGGGSGGGGSGGGGSQDSTSDLIPAPPLSKVPLQQNFQDNQFQGKWYVVGRAGNVGLREDKDPPKMWATIYELKEDKSYDVTNVRFARKKCTYSIGTFVPGSQPGEFTLGQIKSEPGGTANLVRVVSTNYNQHAMVFFKEVYQNREIFFIILYGRTKELTSELKENFIRFSKSLGLPENHIVFPVPIDQCIDG

SEQ ID NO: 37 - protein, 216 aa, artificial; identical to SEQ ID NO: 35
  fusion polypeptide light chain

SEQ ID NO: 38 - protein, 641 aa, artificial
  fusion polypeptide heavy chain
QDSTSDLIPAPPLSKVPLQQNFQDNQFQGKWYVVGRAGNVGLREDKDPPKMWATIYELKEDKSYDVTNVRFARKKCTYSIGTFVPGSQPGEFTLGQIKSEPGGTANLVRVVSTNYNQHAMVFFKEVYQNREIFFIILYGRTKELTSELKENFIRFSKSLGLPENHIVFPVPIDQCIDGGGGGSGGGGSGGGGSQVQLQQWGAGLLKPSETLSLTCAVYGGSFSGYYWSWIRQSPEKGLEWIGEINHGGYVTYNPSLESRVTISVDTSKNQFSLKLSSVTAADTAVYYCARDYGPGNYDWYFDLWGRGTLVTVSSASTKGPSVFPLAPCSRSTSESTAALGCLVKDYFPEPVTVSWNSGALTSGVHTFPAVLQSSGLYSLSSVVTVPSSSLGTKTYTCNVDHKPSNTKVDKRVESKYGPPCPPCPAPEFLGGPSVFLFPPKPKDTLMISRTPEVTCVVVDVSQEDPEVQFNWYVDGVEVHNAKTKPREEQFNSTYRVVSVLTVLHQDWLNGKEYKCKVSNKGLPSSIEKTISKAKGQPREPQVYTLPPSQEEMTKNQVSLTCLVKGFYPSDIAVEWESNGQPENNYKTTPPVLDSDGSFFLYSRLTVDKSRWQEGNVFSCSVMHEALHNHYTQKSLSLSLGK

SEQ ID NO: 39 - protein, 216 aa, artificial; identical to SEQ ID NO: 35
  fusion polypeptide light chain

SEQ ID NO: 40 - protein, 448 aa, artificial; identical to SEQ ID NO: 34
  fusion polypeptide heavy chain

SEQ ID NO: 41 - protein, 409 aa, artificial
  fusion polypeptide light chain
QDSTSDLIPAPPLSKVPLQQNFQDNQFQGKWYVVGRAGNVGLREDKDPPKMWATIYELKEDKSYDVTNVRFARKKCTYSIGTFVPGSQPGEFTLGQIKSEPGGTANLVRVVSTNYNQHAMVFFKEVYQNREIFFIILYGRTKELTSELKENFIRFSKSLGLPENHIVFPVPIDQCIDGGGGGSGGGGSGGGGSEIVLTQSPATLSLSPGERATLSCRASQSVSSYLAWYQQKPGQAPRLLIYDASNRATGIPARFSGSGSGTDFTLTISSLEPEDFAVYYCQQRSNWPPALTFGGGTKVEIKRTVAAPSVFIFPPSDEQLKSGTASVVCLLNNFYPREAKVQWKVDNALQSGNSQESVTEQDSKDSTYSLSSTLTLSKADYEKHKVYACEVTHQGLSSPVTKSFNRGEC

SEQ ID NO: 42 - protein, 448 aa, artificial; identical to SEQ ID NO: 34
  fusion polypeptide heavy chain

SEQ ID NO: 43 - protein, 408 aa, artificial
  fusion polypeptide light chain
EIVLTQSPATLSLSPGERATLSCRASQSVSSYLAWYQQKPGQAPRLLIYDASNRATGIPARFSGSGSGTDFTLTISSLEPEDFAVYYCQQRSNWPPALTFGGGTKVEIKRTVAAPSVFIFPPSDEQLKSGTASVVCLLNNFYPREAKVQWKVDNALQSGNSQESVTEQDSKDSTYSLSSTLTLSKADYEKHKVYACEVTHQGLSSPVTKSFNRGECGGGGSGGGGSGGGGSQDSTSDLIPAPPLSKVPLQQNFQDNQFQGKWYVVGRAGNVGLREDKDPPKMWATIYELKEDKSYDVTNVRFARKKCTYSIGTFVPGSQPGEFTLGQIKSEPGGTANLVRVVSTNYNQHAMVFFKEVYQNREIFFIILYGRTKELTSELKENFIRFSKSLGLPENHIVFPVPIDQCID

SEQ ID NO: 44 - protein, 615 aa, artificial
  fusion polypeptide
QDSTSDLIPAPPLSKVPLQQNFQDNQFQGKWYVVGRAGNVGLREDKDPPKMWATIYELKEDKSYDVTNVRFARKKCTYSIGTFVPGSQPGEFTLGQIKSEPGGTANLVRVVSTNYNQHAMVFFKEVYQNREIFFIILYGRTKELTSELKENFIRFSKSLGLPENHIVFPVPIDQCIDGGGGGSGGGGSGGGGSESKYGPPCPPCPAPEAAGGPSVFLFPPKPKDTLMISRTPEVTCVVVDVSQEDPEVQFNWYVDGVEVHNAKTKPREEQFNSTYRVVSVLTVLHQDWLNGKEYKCKVSNKGLPSSIEKTISKAKGQPREPQVYTLPPSQEEMTKNQVSLTCLVKGFYPSDIAVEWESNGQPENNYKTTPPVLDSDGSFFLYSRLTVDKSRWQEGNVFSCSVMHEALHNHYTQKSLSLSLGKGGGGSGGGGSGGGGSQDSTSDLIPAPPLSKVPLQQNFQDNQFHGKWYVVGQAGNIRLREDKDPIKMMATIYELKEDKSYDVTMVKFDDKKCMYDIWTFVPGSQPGEFTLGKIKSFPGHTSSLVRVVSTNYNQHAMVFFKFVFQNREEFYITLYGRTKELTSELKENFIRFSKSLGLPENHIVFPVPIDQCIDG

SEQ ID NO: 45 - protein, 610 aa, artificial
  fusion polypeptide
QDSTSDLIPAPPLSKVPLQQNFQDNQFQGKWYVVGRAGNVGLREDKDPPKMWATIYELKEDKSYDVTNVRFARKKCTYSIGTFVPGSQPGEFTLGQIKSEPGGTANLVRVVSTNYNQHAMVFFKEVYQNREIFFIILYGRTKELTSELKENFIRFSKSLGLPENHIVFPVPIDQCIDGGGGGSGGGGSQDSTSDLIPAPPLSKVPLQQNFQDNQFHGKWYVVGQAGNIRLREDKDPIKMMATIYELKEDKSYDVTMVKFDDKKCMYDIWTFVPGSQPGEFTLGKIKSFPGHTSSLVRVVSTNYNQHAMVFFKFVFQNREEFYITLYGRTKELTSELKENFIRFSKSLGLPENHIVFPVPIDQCIDGGGGGSGGGGSGGGGSESKYGPPCPPCPAPEAAGGPSVFLFPPKPKDTLMISRTPEVTCVVVDVSQEDPEVQFNWYVDGVEVHNAKTKPREEQFNSTYRVVSVLTVLHQDWLNGKEYKCKVSNKGLPSSIEKTISKAKGQPREPQVYTLPPSQEEMTKNQVSLTCLVKGFYPSDIAVEWESNGQPENNYKTTPPVLDSDGSFFLYSRLTVDKSRWQEGNVFSCSVMHEALHNHYTQKSLSLSLGK

SEQ ID NO: 46 - protein, 366 aa, artificial
  fusion polypeptide
QDSTSDLIPAPPLSKVPLQQNFQDNQFQGKWYVVGVAGNGMLREDKDPLKMRATIYELKEDKSYDVTSVAFRNKKCHYKIGTFVPGSQPGEFTLGQIKSGPGETSNLVRVVSTNYNQHAMVFFKEVRQNREWFFITLYGRTKELTSELKENFIRFSKSLGLPENHIVFPVPIDQCIDGGGGGSGGGGSQDSTSDLIPAPPLSKVPLQQNFQDNQFHGKWYVVGQAGNIRLREDKDPIKMMATIYELKEDKSYDVTMVKFDDKKCMYDIWTFVPGSQPGEFTLGKIKSFPGHTSSLVRVVSTNYNQHAMVFFKFVFQNREEFYITLYGRTKELTSELKENFIRFSKSLGLPENHIVFPVPIDQCIDG

SEQ ID NO: 47 - protein, 554 aa, artificial
  fusion polypeptide
QDSTSDLIPAPPLSKVPLQQNFQDNQFQGKWYVVGVAGNGMLREDKDPLKMRATIYELKEDKSYDVTSVAFRNKKCHYKIGTFVPGSQPGEFTLGQIKSGPGETSNLVRVVSTNYNQHAMVFFKEVRQNREWFFITLYGRTKELTSELKENFIRFSKSLGLPENHIVFPVPIDQCIDGGGGGSGGGGSQDSTSDLIPAPPLSKVPLQQNFQDNQFHGKWYVVGQAGNIRLREDKDPIKMMATIYELKEDKSYDVTMVKFDDKKCMYDIWTFVPGSQPGEFTLGKIKSFPGHTSSLVRVVSTNYNQHAMVFFKFVFQNREEFYITLYGRTKELTSELKENFIRFSKSLGLPENHIVFPVPIDQCIDGGGGGSGGGGSQDSTSDLIPAPPLSKVPLQQNFQDNQFHGKWYVVGQAGNIRLREDKDPIKMMATIYELKEDKSYDVTMVKFDDKKCMYDIWTFVPGSQPGEFTLGKIKSFPGHTSSLVRVVSTNYNQHAMVFFKFVFQNREEFYITLYGRTKELTSELKENFIRFSKSLGLPENHIVFPVPIDQCIDG

SEQ ID NO: 48 - protein, 11 aa, artificial
  peptide linker
GGGGGSGGGGS

SEQ ID NO: 49 - protein, 15 aa, artificial
  peptide linker
GGGGSGGGGSGGGGS

SEQ ID NO: 50 - protein, 10 aa, artificial
  Strep tag
SAWSHPQFEK

SEQ ID NO: 51 - protein, 442 aa, artificial
  antibody heavy chain
EVQLVQSGAEVKKPGESLRISCKGSGYSFSTYWISWVRQMPGKGLEWMGKIYPGDSYTNYSPSFQGQVTISADKSISTAYLQWSSLKASDTAMYYCARGYGIFDYWGQGTLVTVSSASTKGPSVFPLAPCSRSTSESTAALGCLVKDYFPEPVTVSWNSGALTSGVHTFPAVLQSSGLYSLSSVVTVPSSNFGTQTYTCNVDHKPSNTKVDKTVERKCCVECPPCPAPPVAGPSVFLFPPKPKDTLMISRTPEVTCVVVDVSHEDPEVQFNWYVDGVEVHNAKTKPREEQFNSTFRVVSVLTVVHQDWLNGKEYKCKVSNKGLPAPIEKTISKTKGQPREPQVYTLPPSREEMTKNQVSLTCLVKGFYPSDIAVEWESNGQPENNYKTTPPMLDSDGSFFLYSKLTVDKSRWQQGNVFSCSVMHEALHNHYTQKSLSLSPGK

SEQ ID NO: 52 - protein, 214 aa, artificial
  antibody light chain
SYELTQPPSVSVSPGQTASITCSGDNIGDQYAHWYQQKPGQSPVLVIYQDKNRPSGIPERFSGSNSGNTATLTISGTQAMDEADYYCATYTGFGSLAVFGGGTKLTVLGQPKAAPSVTLFPPSSEELQANKATLVCLISDFYPGAVTVAWKADSSPVKAGVETTTPSKQSNNKYAASSYLSLTPEQWKSHRSYSCQVTHEGSTVEKTVAPTECS

SEQ ID NO: 53 - protein, 635 aa, artificial
  fusion polypeptide heavy chain
EVQLVQSGAEVKKPGESLRISCKGSGYSFSTYWISWVRQMPGKGLEWMGKIYPGDSYTNYSPSFQGQVTISADKSISTAYLQWSSLKASDTAMYYCARGYGIFDYWGQGTLVTVSSASTKGPSVFPLAPCSRSTSESTAALGCLVKDYFPEPVTVSWNSGALTSGVHTFPAVLQSSGLYSLSSVVTVPSSNFGTQTYTCNVDHKPSNTKVDKTVERKCCVECPPCPAPPVAGPSVFLFPPKPKDTLMISRTPEVTCVVVDVSHEDPEVQFNWYVDGVEVHNAKTKPREEQFNSTFRVVSVLTVVHQDWLNGKEYKCKVSNKGLPAPIEKTISKTKGQPREPQVYTLPPSREEMTKNQVSLTCLVKGFYPSDIAVEWESNGQPENNYKTTPPMLDSDGSFFLYSKLTVDKSRWQQGNVFSCSVMHEALHNHYTQKSLSLSPGKGGGGSGGGGSGGGGSQDSTSDLIPAPPLSKVPLQQNFQDNQFQGKWYVVGRAGNVGLREDKDPPKMWATIYELKEDKSYDVTNVRFARKKCTYSIGTFVPGSQPGEFTLGQIKSEPGGTANLVRVVSTNYNQHAMVFFKEVYQNREIFFIILYGRTKELTSELKENFIRFSKSLGLPENHIVFPVPIDQCIDG

SEQ ID NO: 54 - protein, 214 aa, artificial; identical to SEQ ID NO: 52
  fusion polypeptide light chain

SEQ ID NO: 55 - DNA, 1344 bp, artificial
  antibody heavy chain
caggtccagctgcagcagtggggggctggtctgctgaagccaagtgaaactctgtcactgacctgcgctgtgtacggcggatcattctccggctactattggtcttggatcagacagagtcccgagaaaggcctggaatggatcggagagattaaccacgggggttacgtgacctataatcctagcctggagtctagggtgaccatttccgtcgacacaagcaagaaccagttctctctgaaactgtccagcgtgacagccgctgacactgcagtctactattgtgccagggattatggccccggaaattacgactggtattttgatctgtgggggcggggtaccctggtgacagtctcgagcgctagcaccaagggcccctccgtgttccccctggccccttgctcccggtccacctccgagtctaccgccgctctgggctgcctggtgaaagactacttccccgagcctgtgaccgtgagctggaactctggcgccctgacctccggcgtgcacaccttccctgccgtgctgcaatcctccggcctgtactccctgtcctccgtggtgacagtgccctcctccagcctgggcaccaagacctacacctgtaacgtggaccacaagccctccaacaccaaggtggacaagcgggtggaatctaaatacggccctccctgccccccctgccctgcccctgaatttctgggcggaccttccgtgtttctgttccccccaaagcccaaggacaccctgatgatctcccggacccccgaagtgacctgcgtggtggtggacgtgtcccaggaagatccagaggtgcagttcaactggtatgttgacggcgtggaagtgcacaacgccaagaccaagcccagagaggaacagttcaactccacctaccgggtggtgtccgtgctgaccgtgctgcaccaggactggctgaacggcaaagagtacaagtgcaaggtgtccaacaagggcctgccctccagcatcgaaaagaccatctccaaggccaagggccagccccgcgagccccaggtgtacaccctgccccctagccaggaagagatgaccaagaaccaggtgtccctgacctgtctggtgaaaggcttctacccctccgacattgccgtggaatgggagtccaacggccagcccgagaacaactacaagaccaccccccctgtgctggactccgacggctccttcttcctgtactctcggctgacagtggataagtcccggtggcaggaaggcaacgtgttctcctgcagcgtgatgcacgaggccctgcacaaccactatacccagaagtccctgtccctgagcctgggcaag

SEQ ID NO: 56 - DNA, 648 bp, artificial
  antibody light chain
gagattgtcctgacccagtcccccgcaacactgtcactgtcccccggcgagagggctactctgagttgccgggcaagccagtctgtgtccagctacctggcctggtatcagcagaagccagggcaggctcccagactgctgatctacgacgcatctaacagagccaccggaattcctgcccgcttctcgggttcaggctccggaacagactttaccctgacaatctctagtctggagccagaagatttcgcagtctactattgtcagcagcgaagcaattggccccctgctctgacttttggcggagggaccaaggtggagatcaagcgtacggtcgcggcgccttctgtgttcattttccccccatctgatgaacagctgaaatctggcactgcttctgtggtctgtctgctgaacaacttctaccctagagaggccaaagtccagtggaaagtggacaatgctctgcagagtgggaattcccaggaatctgtcactgagcaggactctaaggatagcacatactccctgtcctctactctgacactgagcaaggctgattacgagaaacacaaagtgtacgcctgtgaagtcacacatcaggggctgtctagtcctgtgaccaaatccttcaataggggagagtgc

SEQ ID NO: 57 - DNA, 1923 bp, artificial
  fusion polypeptide heavy chain
caggtccagctgcagcagtggggggctggtctgctgaagccaagtgaaactctgtcactgacctgcgctgtgtacggcggatcattctccggctactattggtcttggatcagacagagtcccgagaaaggcctggaatggatcggagagattaaccacgggggttacgtgacctataatcctagcctggagtctagggtgaccatttccgtcgacacaagcaagaaccagttctctctgaaactgtccagcgtgacagccgctgacactgcagtctactattgtgccagggattatggccccggaaattacgactggtattttgatctgtgggggcggggtaccctggtgacagtctcgagcgctagcaccaagggcccctccgtgttccccctggccccttgctcccggtccacctccgagtctaccgccgctctgggctgcctggtgaaagactacttccccgagcctgtgaccgtgagctggaactctggcgccctgacctccggcgtgcacaccttccctgccgtgctgcaatcctccggcctgtactccctgtcctccgtggtgacagtgccctcctccagcctgggcaccaagacctacacctgtaacgtggaccacaagccctccaacaccaaggtggacaagcgggtggaatctaaatacggccctccctgccccccctgccctgcccctgaatttctgggcggaccttccgtgtttctgttccccccaaagcccaaggacaccctgatgatctcccggacccccgaagtgacctgcgtggtggtggacgtgtcccaggaagatccagaggtgcagttcaactggtatgttgacggcgtggaagtgcacaacgccaagaccaagcccagagaggaacagttcaactccacctaccgggtggtgtccgtgctgaccgtgctgcaccaggactggctgaacggcaaagagtacaagtgcaaggtgtccaacaagggcctgccctccagcatcgaaaagaccatctccaaggccaagggccagccccgcgagccccaggtgtacaccctgccccctagccaggaagagatgaccaagaaccaggtgtccctgacctgtctggtgaaaggcttctacccctccgacattgccgtggaatgggagtccaacggccagcccgagaacaactacaagaccaccccccctgtgctggactccgacggctccttcttcctgtactctcggctgacagtggataagtcccggtggcaggaaggcaacgtgttctcctgcagcgtgatgcacgaggccctgcacaaccactatacccagaagtccctgtccctgagcctgggcaagggcggtggaggatccgggggtgggggaagcggcggaggaggtagccaggactccactagcgatctgatcccggctccccctctgagtaaggtgcccctgcaacaaaacttccaagacaatcagtttcagggcaaatggtacgtggtcgggagagctggtaacgtgggactgcgagaggacaaggacccccccaaaatgtgggccaccatctacgagctgaaggaagacaaaagctatgatgtgacaaatgtcaggttcgcacggaagaaatgcacttactcaatcggcaccttcgtgcccggctcccagcctggggagtttacactgggccagattaagagcgaacctggcggaacagccaacctggtgcgggtggtctctactaactataatcagcacgctatggtgttctttaaagaggtctaccagaaccgagaaatcttctttatcatcctgtacggccgtaccaaggagctgacatccgagctgaaagaaaacttcatccgcttttctaagagtctgggactgccagaaaatcatattgtgtttcctgtcccaatcgaccagtgtattgatggg

SEQ ID NO: 58 - DNA, 648 bp, artificial; identical to SEQ ID NO: 56
  fusion polypeptide light chain

SEQ ID NO: 59 - DNA, 1923 bp, artificial
  fusion polypeptide heavy chain
caggactccactagcgatctgatcccggctccccctctgagtaaggtgcccctgcaacaaaacttccaagacaatcagtttcagggcaaatggtacgtggtcgggagagctggtaacgtgggactgcgagaggacaaggacccccccaaaatgtgggccaccatctacgagctgaaggaagacaaaagctatgatgtgacaaatgtcaggttcgcacggaagaaatgcacttactcaatcggcaccttcgtgcccggctcccagcctggggagtttacactgggccagattaagagcgaacctggcggaacagccaacctggtgcgggtggtctctactaactataatcagcacgctatggtgttctttaaagaggtctaccagaaccgagaaatcttctttatcatcctgtacggccgtaccaaggagctgacatccgagctgaaagaaaacttcatccgcttttctaagagtctgggactgccagaaaatcatattgtgtttcctgtcccaatcgaccagtgtattgatgggggcggtggaggatccgggggtgggggaagcggcggaggaggtagccaggtgcaactgcaacaatggggcgcaggcttgttgaagccctctgagacactgagtcttacctgtgctgtgtacggtggcagcttttccggatactattggtcctggattcggcagtctccagagaaaggactggaatggatcggggagatcaatcatggaggctacgttacttacaatccctccctggagagtcgagtgacgatctctgtggatacatctaaaaaccagttttctctcaagctgagttctgttacagcggctgacaccgccgtatactattgtgcgcgggactatggccctggcaactacgactggtactttgacctgtgggggagaggcacgctggtgacagtctcgagcgctagcaccaagggcccctccgtgttccccctggccccttgctcccggtccacctccgagtctaccgccgctctgggctgcctggtgaaagactacttccccgagcctgtgaccgtgagctggaactctggcgccctgacctccggcgtgcacaccttccctgccgtgctgcaatcctccggcctgtactccctgtcctccgtggtgacagtgccctcctccagcctgggcaccaagacctacacctgtaacgtggaccacaagccctccaacaccaaggtggacaagcgggtggaatctaaatacggccctccctgccccccctgccctgcccctgaatttctgggcggaccttccgtgtttctgttccccccaaagcccaaggacaccctgatgatctcccggacccccgaagtgacctgcgtggtggtggacgtgtcccaggaagatccagaggtgcagttcaactggtatgttgacggcgtggaagtgcacaacgccaagaccaagcccagagaggaacagttcaactccacctaccgggtggtgtccgtgctgaccgtgctgcaccaggactggctgaacggcaaagagtacaagtgcaaggtgtccaacaagggcctgccctccagcatcgaaaagaccatctccaaggccaagggccagccccgcgagccccaggtgtacaccctgccccctagccaggaagagatgaccaagaaccaggtgtccctgacctgtctggtgaaaggcttctacccctccgacattgccgtggaatgggagtccaacggccagcccgagaacaactacaagaccaccccccctgtgctggactccgacggctccttcttcctgtactctcggctgacagtggataagtcccggtggcaggaaggcaacgtgttctcctgcagcgtgatgcacgaggccctgcacaaccactatacccagaagtccctgtccctgagcctgggcaag

SEQ ID NO: 60 - DNA, 648 bp, artificial; identical to SEQ ID NO: 56
  fusion polypeptide light chain

SEQ ID NO: 61 - DNA, 1344 bp, artificial; identical to SEQ ID NO: 55
  fusion polypeptide heavy chain

SEQ ID NO: 62 - DNA, 1227 bp, artificial
  fusion polypeptide light chain
caggactccactagcgatctgatcccggctccccctctgagtaaggtgcccctgcaacaaaacttccaagacaatcagtttcagggcaaatggtacgtggtcgggagagctggtaacgtgggactgcgagaggacaaggacccccccaaaatgtgggccaccatctacgagctgaaggaagacaaaagctatgatgtgacaaatgtcaggttcgcacggaagaaatgcacttactcaatcggcaccttcgtgcccggctcccagcctggggagtttacactgggccagattaagagcgaacctggcggaacagccaacctggtgcgggtggtctctactaactataatcagcacgctatggtgttctttaaagaggtctaccagaaccgagaaatcttctttatcatcctgtacggccgtaccaaggagctgacatccgagctgaaagaaaacttcatccgcttttctaagagtctgggactgccagaaaatcatattgtgtttcctgtcccaatcgaccagtgtattgatgggggcggtggaggatccgggggtgggggaagcggcggaggaggtagcgagattgtccttacacagtcaccagccaccctgtccttgtcacccggtgagcgcgccacactgtcctgccgggcatcacaaagcgttagctcctacttggcatggtaccagcagaagcctggacaggccccaaggctgctgatctatgatgctagcaacagggccaccggcattcccgcccgtttctctggtagtgggagcggcactgactttacattgacaatctcttcattggagcccgaggactttgctgtgtactactgtcagcagcggagcaactggcctcccgccctgaccttcggcgggggcacaaaggtggagattaagcgtacggtcgcggcgccttctgtgttcattttccccccatctgatgaacagctgaaatctggcactgcttctgtggtctgtctgctgaacaacttctaccctagagaggccaaagtccagtggaaagtggacaatgctctgcagagtgggaattcccaggaatctgtcactgagcaggactctaaggatagcacatactccctgtcctctactctgacactgagcaaggctgattacgagaaacacaaagtgtacgcctgtgaagtcacacatcaggggctgtctagtcctgtgaccaaatccttcaataggggagagtgc

SEQ ID NO: 63 - DNA, 1029 bp, artificial
  fusion polypeptide heavy chain
tggtattttgatctgtgggggcggggtaccctggtgacagtctcgagcgctagcaccaagggcccctccgtgttccccctggccccttgctcccggtccacctccgagtctaccgccgctctgggctgcctggtgaaagactacttccccgagcctgtgaccgtgagctggaactctggcgccctgacctccggcgtgcacaccttccctgccgtgctgcaatcctccggcctgtactccctgtcctccgtggtgacagtgccctcctccagcctgggcaccaagacctacacctgtaacgtggaccacaagccctccaacaccaaggtggacaagcgggtggaatctaaatacggccctccctgccccccctgccctgcccctgaatttctgggcggaccttccgtgtttctgttccccccaaagcccaaggacaccctgatgatctcccggacccccgaagtgacctgcgtggtggtggacgtgtcccaggaagatccagaggtgcagttcaactggtatgttgacggcgtggaagtgcacaacgccaagaccaagcccagagaggaacagttcaactccacctaccgggtggtgtccgtgctgaccgtgctgcaccaggactggctgaacggcaaagagtacaagtgcaaggtgtccaacaagggcctgccctccagcatcgaaaagaccatctccaaggccaagggccagccccgcgagccccaggtgtacaccctgccccctagccaggaagagatgaccaagaaccaggtgtccctgacctgtctggtgaaaggcttctacccctccgacattgccgtggaatgggagtccaacggccagcccgagaacaactacaagaccaccccccctgtgctggactccgacggctccttcttcctgtactctcggctgacagtggataagtcccggtggcaggaaggcaacgtgttctcctgcagcgtgatgcacgaggccctgcacaaccactatacccagaagtccctgtccctgagcctgggcaag

SEQ ID NO: 64 - DNA, 1224 bp, artificial
  fusion polypeptide light chain
gagattgtcctgacccagtcccccgcaacactgtcactgtcccccggcgagagggctactctgagttgccgggcaagccagtctgtgtccagctacctggcctggtatcagcagaagccagggcaggctcccagactgctgatctacgacgcatctaacagagccaccggaattcctgcccgcttctcgggttcaggctccggaacagactttaccctgacaatctctagtctggagccagaagatttcgcagtctactattgtcagcagcgaagcaattggccccctgctctgacttttggcggagggaccaaggtggagatcaagcgtacggtcgcggcgccttctgtgttcattttccccccatctgatgaacagctgaaatctggcactgcttctgtggtctgtctgctgaacaacttctaccctagagaggccaaagtccagtggaaagtggacaatgctctgcagagtgggaattcccaggaatctgtcactgagcaggactctaaggatagcacatactccctgtcctctactctgacactgagcaaggctgattacgagaaacacaaagtgtacgcctgtgaagtcacacatcaggggctgtctagtcctgtgaccaaatccttcaataggggagagtgcggcggcggaggatccgggggtgggggaagcggcggaggaggtagccaggactccactagcgatctgatcccggctccccctctgagtaaggtgcccctgcaacaaaacttccaagacaatcagtttcagggcaaatggtacgtggtcgggagagctggtaacgtgggactgcgagaggacaaggacccccccaaaatgtgggccaccatctacgagctgaaggaagacaaaagctatgatgtgacaaatgtcaggttcgcacggaagaaatgcacttactcaatcggcaccttcgtgcccggctcccagcctggggagtttacactgggccagattaagagcgaacctggcggaacagccaacctggtgcgggtggtctctactaactataatcagcacgctatggtgttctttaaagaggtctaccagaaccgagaaatcttctttatcatcctgtacggccgtaccaaggagctgacatccgagctgaaagaaaacttcatccgcttttctaagagtctgggactgccagaaaatcatattgtgtttcctgtcccaatcgaccagtgtattgat

SEQ ID NO: 65 - DNA, 1845 bp, artificial
  fusion polypeptide
caggactccactagcgatctgatcccggctccccctctgagtaaggtgcccctgcaacaaaacttccaagacaatcagtttcagggcaaatggtacgtggtcgggagagctggtaacgtgggactgcgagaggacaaggacccccccaaaatgtgggccaccatctacgagctgaaggaagacaaaagctatgatgtgacaaatgtcaggttcgcacggaagaaatgcacttactcaatcggcaccttcgtgcccggctcccagcctggggagtttacactgggccagattaagagcgaacctggcggaacagccaacctggtgcgggtggtctctactaactataatcagcacgctatggtgttctttaaagaggtctaccagaaccgagaaatcttctttatcatcctgtacggccgtaccaaggagctgacatccgagctgaaagaaaacttcatccgcttttctaagagtctgggactgccagaaaatcatattgtgtttcctgtcccaatcgaccagtgtattgatgggggcggtggaggatccgggggtgggggaagcggcggaggaggtagcgaatcgaaatacggccctccctgccccccctgccctgcccctgaagctgcgggcggaccttccgtgtttctgttccccccaaagcccaaggacaccctgatgatctcccggacccccgaagtgacctgcgtggtggtggacgtgtcccaggaagatccagaggtgcagttcaactggtatgttgacggcgtggaagtgcacaacgccaagaccaagcccagagaggaacagttcaactccacctaccgggtggtgtccgtgctgaccgtgctgcaccaggactggctgaacggcaaagagtacaagtgcaaggtgtccaacaagggcctgccctccagcatcgaaaagaccatctccaaggccaagggccagccccgcgagccccaggtgtacaccctgccccctagccaggaagagatgaccaagaaccaggtgtccctgacctgtctggtgaaaggcttctacccctccgacattgccgtggaatgggagtccaacggccagcccgagaacaactacaagaccaccccccctgtgctggactccgacggctccttcttcctgtactctcggctgacagtggataagtcccggtggcaggaaggcaatgtgttctcctgcagcgtgatgcacgaggccctgcacaaccactatacccagaagtccctgtccctgagcctgggcaagggcggtggaggatccgggggtgggggaagcggcggaggaggtagccaggactctactagtgatctgatcccggcaccgccactgtcaaaagtccctctgcaacaaaactttcaagacaatcagtttcacggcaaatggtatgtggtcggccaggccggaaacattaggctgcgggaggacaaggaccccatcaaaatgatggctaccatctacgagctgaaggaagacaaatcttatgatgtgacaatggtcaagttcgacgataagaaatgcatgtacgacatctggaccttcgtgcccggctcccagccgggagagttcaccctgggcaagatcaagtccttccccggccacacttccagcctggtccgcgtggtctcgaccaactataatcagcatgctatggtgttcttcaagttcgtctttcagaatagagaggagttctacatcacactgtatggacgcaccaaggagctgacaagcgagctgaaagaaaacttcatcaggttttcaaagtccctggggctgcccgaaaatcatatcgtgttcccagtccccatcgaccagtgtattgatggt

SEQ ID NO: 66 - DNA, 1830 bp, artificial
  fusion polypeptide
caggactctactagtgatctgattccagcccctccactgagtaaggtgcccctgcagcagaacttccaggacaatcagtttcagggcaagtggtatgtcgtgggaagagcaggaaacgtgggactgcgtgaggacaaggaccctccaaaaatgtgggccactatctacgagctgaaggaagacaaatcctatgatgtgaccaatgtcagattcgctcgcaagaaatgtacatactccatcggaactttcgtgcctggaagccagccaggggagtttaccctggggcagattaagtcagaaccaggcggaaccgccaacctggtgcgagtggtctccacaaactataatcagcacgctatggtgttctttaaagaggtctaccagaacagggaaatcttctttatcatcctgtacggccggaccaaggagctgacatccgagctgaaagaaaacttcatccgtttttcaaagtccctgggactgcccgaaaatcatatcgtgttccccgtccctatcgaccagtgcattgatgggggtggcggagggtccggtggcggagggagccaggacagcacatcggatctgatcccggcaccgccactgtcgaaagtcccactgcaacaaaattttcaagacaatcagtttcacggcaagtggtacgtggtcggtcaggctggcaacattaggctgcgggaggacaaggaccccatcaagatgatggcaacaatctacgagctgaaggaggacaaatcttatgatgtgactatggtcaagttcgacgataagaaatgtatgtacgacatctggaccttcgtgcccggctcccagcctggcgagttcacactgggcaagatcaagtccttccccggccacacttccagcctagtcagagtggtcagcaccaactataatcagcatgctatggtgttctttaagttcgtctttcagaatagagaggagttctacatcaccctgtatggccgcactaaggagctgacctctgagctgaaagagaatttcatccggtttagtaagtcactgggcctgcctgagaatcatatcgtgttcccagtccccattgatcagtgcattgatggtggcggagggggatccgggggtgggggaagcggcggaggaggtagcgaatcgaaatacggccctccctgccccccctgccctgcccctgaagctgcgggcggaccttccgtgtttctgttccccccaaagcccaaggacaccctgatgatctcccggacccccgaagtgacctgcgtggtggtggacgtgtcccaggaagatccagaggtgcagttcaactggtatgttgacggcgtggaagtgcacaacgccaagaccaagcccagagaggaacagttcaactccacctaccgggtggtgtccgtgctgaccgtgctgcaccaggactggctgaacggcaaagagtacaagtgcaaggtgtccaacaagggcctgccctccagcatcgaaaagaccatctccaaggccaagggccagccccgcgagccccaggtgtacaccctgccccctagccaggaagagatgaccaagaaccaggtgtccctgacctgtctggtgaaaggcttctacccctccgacattgccgtggaatgggagtccaacggccagcccgagaacaactacaagaccaccccccctgtgctggactccgacggctccttcttcctgtactctcggctgacagtggataagtcccggtggcaggaaggcaatgtgttctcctgcagcgtgatgcacgaggccctgcacaaccactatacccagaagtccctgtccctgagcctgggcaag

SEQ ID NO: 67 - DNA, 1098 bp, artificial
  fusion polypeptide
caggactccacctcagacctgatcccagccccacctctgagcaaggtccctctgcagcagaacttccaggacaaccaattccaagggaaatggtatgtcgtgggcgttgccggaaatggtatgctgcgtgaggataaggatccgcttaaaatgagggcgaccatttacgagttgaaagaagataaatcatatgacgtcaccagtgtggcttttcggaataagaaatgccattacaagattgggacctttgtgccggggagccagccgggcgagtttactttaggccagattaaaagtggtccgggcgagacatcaaatttggtccgcgtcgtgagcaccaactacaaccagcatgccatggtgttcttcaaggaggtgaggcagaaccgcgagtggttttttatcacactgtacgggcgcacgaaagaactgacaagcgagctgaaggaaaattttatccgcttttccaaatctctgggcctccctgaaaaccacatcgtcttccctgtcccaatcgaccagtgtatcgacggcggtggtggtggttctggtggtggtggatcgcaggactccacctcagacctgatcccagccccacctctgagcaaggtccctctgcagcagaacttccaggacaaccaattccatgggaaatggtacgttgtcgggcaggccggaaatattaggctgcgtgaggataaggatccgattaaaatgatggcgaccatttacgagttgaaagaagataaatcatatgacgtcaccatggtgaagtttgatgataagaaatgcatgtacgatatttggacctttgtgccggggagccagccgggcgagtttactttaggcaagattaaaagttttccgggccatacatcatcgttggtccgcgtcgtgagcaccaactacaaccagcatgccatggtgttcttcaagtttgtgtttcagaaccgcgaggagttttatatcacactgtacgggcgcacgaaagaactgacaagcgagctgaaggaaaattttatccgcttttccaaatctctgggcctccctgaaaaccacatcgtcttccctgtcccaatcgaccagtgtatcgacggc

SEQ ID NO: 68 - DNA, 1662 bp, artificial
  fusion polypeptide
caggactccacctcagacctgatcccagccccacctctgagcaaggtccctctgcagcagaacttccaggacaaccaattccaagggaaatggtatgtcgtgggcgttgccggaaatggtatgctgcgtgaggataaggatccgcttaaaatgagggcgaccatttacgagttgaaagaagataaatcatatgacgtcaccagtgtggcttttcggaataagaaatgccattacaagattgggacctttgtgccggggagccagccgggcgagtttactttaggccagattaaaagtggtccgggcgagacatcaaatttggtccgcgtcgtgagcaccaactacaaccagcatgccatggtgttcttcaaggaggtgaggcagaaccgcgagtggttttttatcacactgtacgggcgcacgaaagaactgacaagcgagctgaaggaaaattttatccgcttttccaaatctctgggcctccctgaaaaccacatcgtcttccctgtcccaatcgaccagtgtatcgacggcggtggtggtggttctggtggtggtggatcgcaggactccacctcagacctgatcccagccccacctctgagcaaggtccctctgcagcagaacttccaggacaaccaattccatgggaaatggtacgttgtcgggcaggccggaaatattaggctgcgtgaggataaggatccgattaaaatgatggcgaccatttacgagttgaaagaagataaatcatatgacgtcaccatggtgaagtttgatgataagaaatgcatgtacgatatttggacctttgtgccggggagccagccgggcgagtttactttaggcaagattaaaagttttccgggccatacatcatcgttggtccgcgtcgtgagcaccaactacaaccagcatgccatggtgttcttcaagtttgtgtttcagaaccgcgaggagttttatatcacactgtacgggcgcacgaaagaactgacaagcgagctgaaggaaaattttatccgcttttccaaatctctgggcctccctgaaaaccacatcgtcttccctgtcccaatcgaccagtgtatcgacggcggcggaggtggctcaggaggtggcggatcccaggactccacctcagacctgatcccagccccacctctgagcaaggtccctctgcagcagaacttccaggacaaccaattccatgggaaatggtacgttgtcgggcaggccggaaatattaggctgcgtgaggataaggatccgattaaaatgatggcgaccatttacgagttgaaagaagataaatcatatgacgtcaccatggtgaagtttgatgataagaaatgcatgtacgatatttggacctttgtgccggggagccagccgggcgagtttactttaggcaagattaaaagttttccgggccatacatcatcgttggtccgcgtcgtgagcaccaactacaaccagcatgccatggtgttcttcaagtttgtgtttcagaaccgcgaggagttttatatcacactgtacgggcgcacgaaagaactgacaagcgagctgaaggaaaattttatccgcttttccaaatctctgggcctccctgaaaaccacatcgtcttccctgtcccaatcgaccagtgtatcgacggc

SEQ ID NO: 69 - DNA, 1326 bp, artificial
  antibody heavy chain
gaggtccagctggtgcagagcggtgccgaagtcaagaagcctggcgagagcctgcggatttcctgcaaaggaagcggatactcattcagcacatactggatctcttgggtcaggcagatgccaggcaagggactggagtggatggggaaaatctaccccggagacagttacactaactattctccgagtttccaaggccaggtcactatcagcgctgataagtcaatttccaccgcctacctgcaatggtccagcctgaaagcctccgacaccgctatgtactattgcgctcgggggtacggtatctttgattattggggccagggaaccctggtgacagtctcgagcgctagcaccaagggcccctccgtgtttcctctggccccttgctccagatccacctccgagtctaccgccgctctgggctgcctcgtgaaggactacttccccgagcctgtgaccgtgtcctggaactctggcgctctgacctctggcgtgcacaccttccctgctgtgctgcagtctagcggcctgtactccctgtcctccgtcgtgaccgtgccctcctctaacttcggcacccagacctacacctgtaacgtggaccacaagccctccaacaccaaggtggacaagaccgtggaacggaagtgctgcgtggaatgccccccttgtcctgcccctcctgtggctggccctagcgtgttcctgttccccccaaagcccaaggacaccctgatgatctcccggacccccgaagtgacctgcgtggtggtggatgtgtcccacgaggaccccgaggtgcagttcaattggtacgtggacggcgtggaagtgcacaacgccaagaccaagcccagagaggaacagttcaactccaccttccgggtggtgtccgtgctgaccgtggtgcatcaggactggctgaacggcaaagagtacaagtgcaaggtgtccaacaagggcctgcctgcccccatcgaaaagaccatctctaagaccaagggacagccccgcgagccccaggtgtacacactgcctccatcacgggaagagatgaccaagaaccaggtgtccctgacctgtctcgtgaaaggcttctacccctccgatatcgccgtggaatgggagtccaacggccagcccgagaacaactacaagaccaccccccccatgctggactccgacggctcattcttcctgtactccaagctgacagtggacaagtcccggtggcagcagggcaacgtgttctcctgctccgtgatgcacgaggccctgcacaaccactacacccagaagtccctgtccctgagccccgggaaa

SEQ ID NO: 70 - DNA, 642 bp, artificial
  antibody light chain
tcctatgaactgacacagcctccttccgtgagcgtgagccctggacagactgcttctattacttgtagcggggataacatcggggatcagtacgcccactggtatcagcagaagcccggacagagtcctgtgctggtcatctaccaggacaaaaacaggccatcaggcattcccgagcggttctccggaagcaactctgggaataccgctacactgactatctccggaacacaggcaatggacgaagccgattactattgcgctacctatacaggtttcggctctctggcagtgtttggcggagggactaagctgaccgtcctgggccagcctaaagcggcgccatccgtcaccctgttccctccctcatccgaggaactgcaggccaataaggctacactggtctgtctgattagcgacttctaccctggggccgtgactgtggcttggaaagccgattcttctcccgtgaaagctggagtggaaacaaccaccccctctaaacagagcaacaacaaatacgctgcctcttcatacctgtccctgacccctgaacagtggaaatctcaccggtcttactcatgccaggtgacacacgagggatcaactgtggagaaaaccgtggctcctaccgaatgttca

SEQ ID NO: 71 - DNA, 1905 bp, artificial
  fusion polypeptide heavy chain
gaggtccagctggtgcagagcggtgccgaagtcaagaagcctggcgagagcctgcggatttcctgcaaaggaagcggatactcattcagcacatactggatctcttgggtcaggcagatgccaggcaagggactggagtggatggggaaaatctaccccggagacagttacactaactattctccgagtttccaaggccaggtcactatcagcgctgataagtcaatttccaccgcctacctgcaatggtccagcctgaaagcctccgacaccgctatgtactattgcgctcgggggtacggtatctttgattattggggccagggaaccctggtgacagtctcgagcgctagcaccaagggcccctccgtgtttcctctggccccttgctccagatccacctccgagtctaccgccgctctgggctgcctcgtgaaggactacttccccgagcctgtgaccgtgtcctggaactctggcgctctgacctctggcgtgcacaccttccctgctgtgctgcagtctagcggcctgtactccctgtcctccgtcgtgaccgtgccctcctctaacttcggcacccagacctacacctgtaacgtggaccacaagccctccaacaccaaggtggacaagaccgtggaacggaagtgctgcgtggaatgccccccttgtcctgcccctcctgtggctggccctagcgtgttcctgttccccccaaagcccaaggacaccctgatgatctcccggacccccgaagtgacctgcgtggtggtggatgtgtcccacgaggaccccgaggtgcagttcaattggtacgtggacggcgtggaagtgcacaacgccaagaccaagcccagagaggaacagttcaactccaccttccgggtggtgtccgtgctgaccgtggtgcatcaggactggctgaacggcaaagagtacaagtgcaaggtgtccaacaagggcctgcctgcccccatcgaaaagaccatctctaagaccaagggacagccccgcgagccccaggtgtacacactgcctccatcacgggaagagatgaccaagaaccaggtgtccctgacctgtctcgtgaaaggcttctacccctccgatatcgccgtggaatgggagtccaacggccagcccgagaacaactacaagaccaccccccccatgctggactccgacggctcattcttcctgtactccaagctgacagtggacaagtcccggtggcagcagggcaacgtgttctcctgctccgtgatgcacgaggccctgcacaaccactacacccagaagtccctgtccctgagccccgggaaaggcggcggaggatccgggggtgggggaagcggcggaggaggtagccaggactccactagcgatctgatcccggctccccctctgagtaaggtgcccctgcaacaaaacttccaagacaatcagtttcagggcaaatggtacgtggtcgggagagctggtaacgtgggactgcgagaggacaaggacccccccaaaatgtgggccaccatctacgagctgaaggaagacaaaagctatgatgtgacaaatgtcaggttcgcacggaagaaatgcacttactcaatcggcaccttcgtgcccggctcccagcctggggagtttacactgggccagattaagagcgaacctggcggaacagccaacctggtgcgggtggtctctactaactataatcagcacgctatggtgttctttaaagaggtctaccagaaccgagaaatcttctttatcatcctgtacggccgtaccaaggagctgacatccgagctgaaagaaaacttcatccgcttttctaagagtctgggactgccagaaaatcatattgtgtttcctgtcccaatcgaccagtgtattgatggg

SEQ ID NO: 72 - DNA, 642 bp, artificial; identical to SEQ ID NO: 70
  fusion polypeptide light chain

SEQ ID NO: 73 - protein, 229 aa, artificial
  IgG4-Fc with mutations
ESKYGPPCPPCPAPEAAGGPSVFLFPPKPKDTLMISRTPEVTCVVVDVSQEDPEVQFNWYVDGVEVHNAKTKPREEQFNSTYRVVSVLTVLHQDWLNGKEYKCKVSNKGLPSSIEKTISKAKGQPREPQVYTLPPSQEEMTKNQVSLTCLVKGFYPSDIAVEWESNGQPENNYKTTPPVLDSDGSFFLYSRLTVDKSRWQEGNVFSCSVMHEALHNHYTQKSLSLSLGK

SEQ ID NO: 74 - protein, 448 aa, artificial; identical to SEQ ID NO: 34
  reference antibody

SEQ ID NO: 75 - protein, 216 aa, reference antibody; identical to SEQ ID NO: 35